European Patent Specification EP 3 653 645 B1, published August 21, 2024. Title: INTERLEUKIN-31 MONOCLONAL ANTIBODY. Applicant: Pfizer Inc. Bammert, Gary F. Dunham, Steven A. The sequence listing filed with the application follows.

SEQUENCE LISTING (78 sequences)

SEQ ID NO: 1 - protein, 5 aa, Mus musculus
YYDIN

SEQ ID NO: 2 - protein, 5 aa, Mus musculus
SYDMS

SEQ ID NO: 3 - protein, 5 aa, Mus musculus
NYGMS

SEQ ID NO: 4 - protein, 17 aa, Mus musculus
WIFPGDGGTKYNETFKG

SEQ ID NO: 5 - protein, 17 aa, Mus musculus
TITSGGGYTYSADSVKG

SEQ ID NO: 6 - protein, 17 aa, Mus musculus
TISYGGSYTYYPDNIKG

SEQ ID NO: 7 - protein, 14 aa, Mus musculus
ARGGTSVIRDAMDY

SEQ ID NO: 8 - protein, 11 aa, Mus musculus
ARQNWVVGLAY

SEQ ID NO: 9 - protein, 11 aa, Mus musculus
VRGYGYDTMDY

SEQ ID NO: 10 - protein, 15 aa, Mus musculus
RASESVDNYGISFMH

SEQ ID NO: 11 - protein, 17 aa, Mus musculus
KSSQSLLNSGNQKNYLA

SEQ ID NO: 12 - protein, 15 aa, Mus musculus
KASQSVSFAGTGLMH

SEQ ID NO: 13 - protein, 7 aa, Mus musculus
RASNLES

SEQ ID NO: 14 - protein, 7 aa, Mus musculus
GASTRES

SEQ ID NO: 15 - protein, 7 aa, Mus musculus
RASNLEA

SEQ ID NO: 16 - protein, 9 aa, Mus musculus
QQSNKDPLT

SEQ ID NO: 17 - protein, 9 aa, Mus musculus
QNDYSYPYT

SEQ ID NO: 18 - protein, 9 aa, Mus musculus
QQSREYPWT

SEQ ID NO: 19 - protein, 111 aa, Mus musculus
DIVLTQSPASLAVSLGQRATISCRASESVDNYGISFMHWYQQKPGQPPKLLIYRASNLESGIPARFSGSGSRTDFTLTINPVETDDVATYYCQQSNKDPLTFGAGTKLELK

SEQ ID NO: 20 - protein, 111 aa, Artificial
  caninized variable light chain mAb sequence, from Mus musculus and Canis
DIVMTQTPLSLSVSPGEPASISCRASESVDNYGISFMHWYQQKPGQPPKLLIYRASNLESGVPDRFSGSGSGTDFTLRISRVEADDAGVYYCQQSNKDPLTFGAGTKLEIK

SEQ ID NO: 21 - protein, 111 aa, Artificial
  caninized variable light chain mAb sequence, from Mus musculus and Canis
DIVMTQTPLSLSVSPGEPASISCRASESVDNYGISFMHWFQQKPGQSPQLLIYRASNLESGVPDRFSGSGSGTDFTLRISRVEADDAGVYYCQQSNKDPLTFGAGTKLEIK

SEQ ID NO: 22 - protein, 113 aa, Mus musculus
DIVMSQSPSSLSVSAGDKVTMSCKSSQSLLNSGNQKNYLAWYQQKPWQPPKLLIYGASTRESGVPDRFTGSGSGTDFTLTISSVQAEDLAVYYCQNDYSYPYTFGGGTKLEIK

SEQ ID NO: 23 - protein, 113 aa, Artificial
  caninized variable light chain mAb sequence, from Mus musculus and Canis
EIVMTQSPASLSLSQEEKVTITCKSSQSLLNSGNQKNYLAWYQQKPGQAPKLLIYGASTRESGVPSRFSGSGSGTDFSFTISSLEPEDVAVYYCQNDYSYPYTFGQGTKLEIK

SEQ ID NO: 24 - protein, 111 aa, Mus musculus
DILLTQSPASLAVSLGQRAIISCKASQSVSFAGTGLMHWYQQKPGQQPKLLIYRASNLEAGVPTRFSGSGSRTDFTLNIHPVEEEDAATYFCQQSREYPWTFGGGTKLEIK

SEQ ID NO: 25 - protein, 111 aa, Artificial
  caninized variable light chain mAb sequence, from Mus musculus and Canis
EIVMTQSPASLSLSQEEKVTITCKASQSVSFAGTGLMHWYQQKPGQAPKLLIYRASNLEAGVPSRFSGSGSGTDFSFTISSLEPEDVAVYYCQQSREYPWTFGQGTKLEIK

SEQ ID NO: 26 - protein, 121 aa, Mus musculus
QVQLQQSGAELVKPGASVKLSCKASGYTFKYYDINWVRQRPEQGLEWIGWIFPGDGGTKYNETFKGKATLTTDKSSSTAYMQLSRLTSEDSAVYFCARGGTSVIRDAMDYWGQGTSVTVSS

SEQ ID NO: 27 - protein, 121 aa, Artificial
  caninized variable heavy chain mAb sequence, from Mus musculus and Canis
EVQLVQSGAEVKKPGASVKVSCKTSGYTFKYYDINWVRQAPGAGLDWMGWIFPGDGGTKYNETFKGRVTLTADTSTSTAYMELSSLRAGDIAVYYCARGGTSVIRDAMDYWGQGTLVTVSS

SEQ ID NO: 28 - protein, 118 aa, Mus musculus
EVKLVESGGGLVKPGGSLKLSCAASGFAFSSYDMSWVRQIPEKRLEWVATITSGGGYTYSADSVKGRFTISRDNARNTLYLQMSSLRSEDTAVYYCARQNWVVGLAYWGQGTLVTVSA

SEQ ID NO: 29 - protein, 118 aa, Artificial
  caninized variable heavy chain mAb sequence, from Mus musculus and Canis
EVQLVESGGDLVKPGGSLRLSCVASGFTFSSYDMSWVRQAPGKGLQWVATITSGGGYTYSADSVKGRFTISRDNARNTLYLQMNSLRSEDTAVYYCARQNWVVGLAYWGQGTLVTVSS

SEQ ID NO: 30 - protein, 118 aa, Mus musculus
EVQLVESGGDLVKPGGSLKLSCAASGFSFSNYGMSWVRQTPDKRLEWVATISYGGSYTYYPDNIKGRFTISRDNAKNTLYLQMSSLKSEDTAMYYCVRGYGYDTMDYWGQGTSVTVSS

SEQ ID NO: 31 - protein, 118 aa, Artificial
  caninized variable heavy chain mAb sequence, from Mus musculus and Canis
EVQLVESGGDLVKPGGSLRLSCVASGFTFSNYGMSWVRQAPGKGLQWVATISYGGSYTYYPDNIKGRFTISRDNAKNTLYLQMNSLRAEDTAMYYCVRGYGYDTMDYWGQGTLVTVSS

SEQ ID NO: 32 - protein, 159 aa, Canis familiaris
MLSHTGPSRFALFLLCSMETLLSSHMAPTHQLPPSDVRKIILELQPLSRGLLEDYQKKETGVPESNRTLLLCLTSDSQPPRLNSSAILPYFRAIRPLSDKNIIDKIIEQLDKLKFQHEPETEISVPADTFECKSFILTILQQFSACLESVFKSLNSGPQ

SEQ ID NO: 33 - DNA, 477 bp, Canis familiaris
atgctctcccacacaggaccatccaggtttgccctgttcctgctctgctctatggaaaccttgctgtcctcccatatggcacccacccatcagctaccaccaagtgatgtacgaaaaatcatcttggaattacagcccttgtcgaggggacttttggaagactatcagaagaaagagacaggggtgccagaatccaaccgtaccttgctgctgtgtctcacctctgattcccaaccaccacgcctcaacagctcagccatcttgccttatttcagggcaatcagaccattatcagataagaacattattgataaaatcatagaacagcttgacaaactcaaatttcaacatgaaccagaaacagaaatttctgtgcctgcagatacttttgaatgtaaaagcttcatcttgacgattttacagcagttctcggcgtgcctggaaagtgtgtttaagtcactaaactctggacctcag

SEQ ID NO: 34 - DNA, 333 bp, Mus musculus
gacattgtgctgacccaatctccagcttctttggctgtgtctctagggcagagggccaccatctcctgcagagccagcgaaagtgttgataattatggcattagttttatgcactggtaccagcagaaaccaggacagccacccaaactcctcatctatcgtgcatccaacctagaatctgggatccctgccaggttcagtggcagtgggtctaggacagacttcaccctcaccattaatcctgtggagactgatgatgttgcaacctattactgtcagcaaagtaataaggatccgctcacgttcggtgctgggaccaagctggagctgaaa

SEQ ID NO: 35 - DNA, 363 bp, Mus musculus
caggttcagctgcagcagtctggagctgaactggtaaagcctggggcttcagtgaagttgtcctgcaaggcttctggctacaccttcaaatactatgatataaactgggtgaggcagaggcctgaacagggacttgagtggattggatggatttttcctggagatggtggtactaagtacaatgagacgttcaagggcaaggccacactgactacagacaaatcctccagcacagcctacatgcagctcagcaggctgacatctgaggactctgctgtctatttctgtgcaagaggggggacttcggtgataagggatgctatggactactggggtcaaggaacctcagtcaccgtctcctca

SEQ ID NO: 36 - DNA, 339 bp, Mus musculus
gacattgtgatgtcacagtctccatcctccctgagtgtgtcagcaggagataaggtcactatgagctgcaagtccagtcagagtctgttaaacagtggaaatcaaaagaactacttggcctggtaccagcagaaaccatggcagcctcctaaactgctgatctacggggcatccactagggaatctggggtccctgatcgcttcacaggcagtggatctggaacagatttcactctcaccatcagcagtgtgcaggctgaagacctggcagtttattactgtcagaatgattatagttatccgtacacgttcggaggggggaccaagctggaaataaaa

SEQ ID NO: 37 - DNA, 354 bp, Mus musculus
gaagtgaagctggtggagtctgggggaggcttagtgaagcctggagggtccctgaaactctcctgtgcagcctctggattcgctttcagcagctatgacatgtcttgggttcgccagattccggaaaagaggctggagtgggtcgcaaccattactagtggtggtggttacacctactctgcagacagtgtgaagggccgattcaccatctccagagacaatgccaggaacaccctgtacctgcaaatgagcagtctgaggtctgaggacacggccgtgtattattgtgcaagacaaaactgggtcgtggggttagcttattggggccaagggactctggtcactgtctctgca

SEQ ID NO: 38 - DNA, 333 bp, Mus musculus
gacattttgctgacccaatctccagcttctttggctgtgtctctagggcagagggccatcatctcctgcaaggccagccaaagtgtcagttttgctggtactggtttaatgcactggtaccaacagaaaccaggacagcaacccaaactcctcatctatcgtgcatccaacctagaagctggggttcctaccaggtttagtggcagtgggtctaggacagacttcaccctcaatatccatcctgtggaggaggaggatgctgcaacctatttctgtcagcaaagcagggaatatccgtggacgttcggtggaggcaccaagctggaaatcaaa

SEQ ID NO: 39 - DNA, 353 bp, Mus musculus
gaggtgcagttggtggagtctgggggagacttagtgaagcctggagggtccctgaaactctcctgtgcagcctctggattctctttcagtaactatggcatgtcttgggttcgccagactccagacaagaggctggagtgggtcgcaaccattagttatggtggtagttacacctactatccagacaatataaaggggcgattcaccatctccagagacaatgccaagaacaccctgtacctgcaaatgagcagtctgaagtctgaggacacagccatgtattactgtgtaagggggtatggttacgatactatggactactggggtcaaggaacctcagtcaccgtctcgag

SEQ ID NO: 40 - protein, 331 aa, Canis familiaris
ASTTAPSVFPLAPSCGSTSGSTVALACLVSGYFPEPVTVSWNSGSLTSGVHTFPSVLQSSGLHSLSSMVTVPSSRWPSETFTCNVVHPASNTKVDKPVFNECRCTDTPPCPVPEPLGGPSVLIFPPKPKDILRITRTPEVTCVVLDLGREDPEVQISWFVDGKEVHTAKTQSREQQFNGTYRVVSVLPIEHQDWLTGKEFKCRVNHIDLPSPIERTISKARGRAHKPSVYVLPPSPKELSSSDTVSITCLIKDFYPPDIDVEWQSNGQQEPERKHRMTPPQLDEDGSYFLYSKLSVDKSRWQQGDPFTCAVMHETLQNHYTDLSLSHSPGK

SEQ ID NO: 41 - DNA, 993 bp, Canis familiaris
gcctccaccacggcgccctcggttttcccactggcccccagctgcgggtccacttccggctccacggtggccctggcctgcctggtgtcaggctacttccccgagcctgtaactgtgtcctggaactccggctccttgaccagcggtgtgcacaccttcccgtccgtcctgcagtcctcagggcttcactccctcagcagcatggtgacagtgccctccagcaggtggcccagcgagaccttcacctgcaacgtggtccacccagccagcaacactaaagtagacaagccagtgttcaatgaatgcagatgcactgatacacccccatgcccagtccctgaacctctgggagggccttcggtcctcatctttcccccgaaacccaaggacatcctcaggattacccgaacacccgaggtcacctgtgtggtgttagatctgggccgtgaggaccctgaggtgcagatcagctggttcgtggatggtaaggaggtgcacacagccaagacccagtctcgtgagcagcagttcaacggcacctaccgtgtggtcagcgtcctccccattgagcaccaggactggctcacagggaaggagttcaagtgcagagtcaaccacatagacctcccgtctcccatcgagaggaccatctctaaggccagagggagggcccataagcccagtgtgtatgtcctgccgccatccccaaaggagttgtcatccagtgacacagtcagcatcacctgcctgataaaagacttctacccacctgacattgatgtggagtggcagagcaatggacagcaggagcccgagaggaagcaccgcatgaccccgccccagctggacgaggacgggtcctacttcctgtacagcaagctctctgtggacaagagccgctggcagcagggagaccccttcacatgtgcggtgatgcatgaaactctacagaaccactacacagatctatccctctcccattctccgggtaaa

SEQ ID NO: 42 - protein, 335 aa, Canis familiaris
ASTTAPSVFPLAPSCGSTSGSTVALACLVSGYFPEPVTVSWNSGSLTSGVHTFPSVLQSSGLYSLSSMVTVPSSRWPSETFTCNVAHPASKTKVDKPVPKRENGRVPRPPDCPKCPAPEMLGGPSVFIFPPKPKDTLLIARTPEVTCVVVDLDPEDPEVQISWFVDGKQMQTAKTQPREEQFNGTYRVVSVLPIGHQDWLKGKQFTCKVNNKALPSPIERTISKARGQAHQPSVYVLPPSREELSKNTVSLTCLIKDFFPPDIDVEWQSNGQQEPESKYRTTPPQLDEDGSYFLYSKLSVDKSRWQRGDTFICAVMHEALHNHYTQESLSHSPGK

SEQ ID NO: 43 - DNA, 1005 bp, Canis familiaris
gcctcaacaactgctcctagcgtgtttcccctggcccctagctgcggaagtacctcaggcagcacagtggccctggcttgtctggtgtctggatatttccctgagccagtgaccgtgagttggaacagcggctctctgacctccggggtgcacacatttccatctgtgctgcagtctagtggcctgtactccctgtcaagcatggtgactgtgccttcctctaggtggccatcagaaactttcacctgcaacgtggcccatcccgccagcaagaccaaagtggacaagcccgtgcctaaaagggagaatggaagggtgccaagaccacctgattgccctaagtgtccagctccagaaatgctgggaggaccaagcgtgttcatctttccacccaagcccaaagacacactgctgattgctagaactcccgaggtgacctgcgtggtggtggacctggatccagaggaccccgaagtgcagatctcctggttcgtggatgggaagcagatgcagacagccaaaactcagcctcgggaggaacagtttaacggaacctatagagtggtgtctgtgctgccaattggacaccaggactggctgaagggcaaacagtttacatgcaaggtgaacaacaaggccctgcctagtccaatcgagaggactatttcaaaagctaggggacaggctcatcagccttccgtgtatgtgctgcctccatcccgggaggaactgtctaagaacacagtgagtctgacttgtctgatcaaagatttctttccccctgacattgatgtggagtggcagagcaatgggcagcaggagccagaatccaagtacagaaccacaccaccccagctggacgaagatggctcctatttcctgtacagtaagctgtcagtggacaaatctaggtggcagcgcggggatacctttatctgcgccgtgatgcacgaggctctgcacaatcattacacacaagaaagtctgtcacatagccccggcaag

SEQ ID NO: 44 - protein, 106 aa, Canis familiaris
RNDAQPAVYLFQPSPDQLHTGSASVVCLLNSFYPKDINVKWKVDGVIQDTGIQESVTEQDKDSTYSLSSTLTMSSTEYLSHELYSCEITHKSLPSTLIKSFQRSEC

SEQ ID NO: 45 - DNA, 318 bp, Canis familiaris
aggaacgacgcccagcctgctgtgtatctgtttcagccctcccctgatcagctgcacactggctctgctagtgtggtgtgtctgctgaacagcttctacccaaaggatatcaatgtgaagtggaaagtggacggcgtgatccaggatactgggattcaggagtccgtgaccgaacaggacaaagattcaacatatagcctgagctccactctgaccatgtctagtaccgagtacctgagccacgaactgtattcctgcgagatcactcataagtccctgccctctaccctgatcaagagcttccagagatcagagtgt

SEQ ID NO: 46 - DNA, 339 bp, Artificial
  nucleotide sequence encoding a caninized variable light chain mAb sequence, from Mus musculus and Canis
gagatcgtgatgacccagagccccgccagcctgagcctgagccaggaagagaaagtcaccatcacatgcaagagcagccagagcctgctgaacagcggcaaccagaagaactacctggcctggtatcagcagaagcccggccaggcccccaagctgctgatctacggcgccagcacccgcgagagcggcgtgccaagcagattttccggcagcggctccggcaccgacttcagcttcaccatcagcagcctggaacccgaggacgtggccgtgtactactgccagaacgactacagctacccctacaccttcggccagggtaccaagctggagatcaag

SEQ ID NO: 47 - DNA, 354 bp, Artificial
  nucleotide sequence encoding a caninized variable heavy chain mAb sequence, from Mus musculus and Canis
gaggtgcagctggtggaatctggcggcgacctggtcaagcctggcggcagcctgagactgagctgtgtggccagcggcttcaccttcagcagctacgacatgagctgggtccgacaggcccctggcaagggactgcagtgggtggccaccatcaccagcggcggaggctacacctacagcgccgacagcgtgaagggccggttcaccatcagccgggacaacgcccggaacaccctgtacctgcagatgaacagcctgcggagcgaggacaccgccgtgtactactgcgccagacagaactgggtcgtgggcctggcctactggggccagggaacactcgtgaccgtctcgagc

SEQ ID NO: 48 - DNA, 333 bp, Artificial
  nucleotide sequence encoding a caninized variable light chain mAb sequence, from Mus musculus and Canis
gagatcgtgatgacccagagccccgccagcctgagcctgagccaggaagagaaagtcaccatcacatgcaaggccagccagagcgtgtccttcgccggcacaggcctgatgcactggtatcagcagaagcccggccaggcccccaagctgctgatctaccgggccagcaacctggaagccggcgtgccaagcagattcagcggcagcggctccggcaccgacttcagcttcaccatcagcagcctcgaacccgaggacgtggccgtgtactactgccagcagagcagagagtacccctggaccttcggccagggtaccaagctggagatcaag

SEQ ID NO: 49 - DNA, 354 bp, Artificial
  nucleotide sequence encoding a caninized variable heavy chain mAb sequence, from Mus musculus and Canis
gaggtgcagctggtggaatctggcggcgacctggtcaagcctggcggcagcctgagactgagctgtgtggccagcggcttcaccttcagcaactacggcatgagctgggtccgacaggcccctggcaagggactgcagtgggtggccaccatcagctacggcggcagctacacctactaccccgacaacatcaagggccggttcaccatcagccgggacaacgccaagaacaccctgtacctgcagatgaacagcctgcgggccgaggacaccgccatgtactactgcgtgcggggctacggctacgacacaatggactactggggccagggcaccctcgtgaccgtctcgagc

SEQ ID NO: 50 - DNA, 333 bp, Artificial
  nucleotide sequence encoding a caninized variable light chain mAb sequence, from Mus musculus and Canis
gatatagtgatgacacaaactcctctcagtctttccgtatcaccgggagaaccggcttccatttcctgtcgggcctcagagtctgtggacaactacgggatatccttcatgcactggtatcagcagaaacccggccagccccctaaactccttatttacagggccagtaatctggaaagcggtgtgcccgatcgatttagcggttccgggagcggcacagatttcaccctgcgaatctctagagttgaagcggatgatgcaggagtatattactgccagcaatccaataaggatccccttacattcggcgcgggtaccaagctggagatcaag

SEQ ID NO: 51 - DNA, 363 bp, Artificial
  nucleotide sequence encoding a caninized variable heavy chain mAb sequence, from Mus musculus and Canis
gaggtgcagctggtgcagtctggcgccgaagtgaagaaacctggcgccagcgtgaaggtgtcctgcaagaccagcggctacaccttcaagtactacgacatcaactgggtccgacaggcccctggcgccggactggattggatgggctggatcttccccggcgacggcggcaccaagtacaacgagacattcaagggcagagtgaccctgaccgccgacaccagcaccagcaccgcctacatggaactgagcagcctgagagccggcgatatcgctgtgtactactgcgccagaggcggcaccagcgtgatccgggacgctatggactactggggccagggcaccctcgtgaccgtctcgagc

SEQ ID NO: 52 - DNA, 333 bp, Artificial
  nucleotide sequence encoding a caninized variable light chain mAb sequence, from Mus musculus and Canis
gacattgttatgactcagacgcccctgagcctgagcgtctcccccggcgagcccgctagtattagttgccgggcatccgagtcagtggacaattatggcatcagctttatgcattggtttcagcagaaaccaggtcagtcccctcaactcctgatttacagagcttccaatctggaatcaggcgttcctgacagatttagcggatcaggctccgggacagatttcaccctgcgcatcagtcgcgtggaagccgatgacgcaggcgtctattattgtcaacagtccaacaaggatccccttacattcggagccggtaccaagctggagatcaag

SEQ ID NO: 53 - protein, 111 aa, Artificial
  caninized variable light chain mAb sequence, from Mus musculus and Canis
DIVMTQTPLSLSVSPGEPASISCRASESVDNYGISFMHWFQQKPGQSPQRLIYRASNLESGVPDRFSGSGSGTDFTLRISRVEADDAGVYYCQQSNKDPLTFGAGTKLEIK

SEQ ID NO: 54 - DNA, 333 bp, Artificial
  nucleotide sequence encoding a caninized variable light chain mAb sequence, from Mus musculus and Canis
gacatcgtgatgacccagacccccctgagcctgagcgtgtcccctggcgagcctgccagcatcagctgcagagccagcgagagcgtggacaactacggcatcagcttcatgcactggttccagcagaagcccggccagagcccccagcggctgatctacagagccagcaacctggaaagcggcgtgcccgatcggtttagcggctctggcagcggcaccgacttcaccctgcggatctctcgggtggaagccgatgacgccggagtgtactactgccagcagagcaacaaggaccccctgacctttggcgccggtaccaagctggagatcaag

SEQ ID NO: 55 - protein, 148 aa, Artificial
  canine IL-31 full length protein encoded by codon-optimized nucleotide sequence
MRGSHHHHHHGSSHMAPTHQLPPSDVRKIILELQPLSRGLLEDYQKKETGVPESNRTLLLCLTSDSQPPRLNSSAILPYFRAIRPLSDKNIIDKIIEQLDKLKFQHEPETEISVPADTFECKSFILTILQQFSACLESVFKSLNSGPQ

SEQ ID NO: 56 - DNA, 444 bp, Artificial
  codon-optimized nucleotide sequence encoding canine IL-31 full-length protein
atgagaggatcccatcaccatcaccaccacggctcatctcatatggctcctactcaccaattaccaccctccgatgtccgtaaaattattctcgaattacaacctttatcccgcggtctgctcgaagattaccaaaaaaaagaaacaggcgtcccagaaagcaaccgtacattactcctttgccttacctccgattcccaaccacctcgtcttaactcatcagccattctcccttatttccgtgccattcgccctctttctgataaaaatattattgacaaaattattgaacaactcgacaaattaaaattccaacacgaacccgaaaccgaaatctccgtacctgccgatacctttgaatgcaaatcctttatcctcactattttacaacaattctccgcatgtctcgaatccgtcttcaaatctctcaattccggtccacag

SEQ ID NO: 57 - protein, 151 aa, Artificial
  amino acid sequence corresponding to canine IL-31 protein with N-terminal truncation (-20N)
MLELQPLSRGLLEDYQKKETGVPESNRTLLLCLTSDSQPPRLNSSAILPYFRAIRPLSDKNIIDKIIEQLDKLKFQHEPETEISVPADTFECKSFILTILQQFSACLESVFKSLNSGPQKGELNSKLEGKPIPNPLLGLDSTRTGHHHHHH

SEQ ID NO: 58 - DNA, 456 bp, Artificial
  nucleotide sequence encoding canine IL-31 protein with N-terminal truncation (-20N)
atgctcgaattacaacctttatcccgcggtctgctcgaagattaccaaaaaaaagaaacaggcgtcccagaaagcaaccgtacattactcctttgccttacctccgattcccaaccacctcgtcttaactcatcagccattctcccttatttccgtgccattcgccctctttctgataaaaatattattgacaaaattattgaacaactcgacaaattaaaattccaacacgaacccgaaaccgaaatctccgtacctgccgatacctttgaatgcaaatcctttatcctcactattttacaacaattctccgcatgtctcgaatccgtcttcaaatctctcaattccggtccacagaagggcgagctcaattcgaagcttgaaggtaagcctatccctaaccctctcctcggtctcgattctacgcgtaccggtcatcatcaccatcaccattga

SEQ ID NO: 59 - protein, 131 aa, Artificial
  amino acid sequence corresponding to canine IL-31 protein with N-terminal truncation (-40N)
MVPESNRTLLLCLTSDSQPPRLNSSAILPYFRAIRPLSDKNIIDKIIEQLDKLKFQHEPETEISVPADTFECKSFILTILQQFSACLESVFKSLNSGPQKGELNSKLEGKPIPNPLLGLDSTRTGHHHHHH

SEQ ID NO: 60 - DNA, 393 bp, Artificial
  nucleotide sequence encoding canine IL-31 protein with N-terminal truncation (-40N)
atggtcccagaaagcaaccgtacattactcctttgccttacctccgattcccaaccacctcgtcttaactcatcagccattctcccttatttccgtgccattcgccctctttctgataaaaatattattgacaaaattattgaacaactcgacaaattaaaattccaacacgaacccgaaaccgaaatctccgtacctgccgatacctttgaatgcaaatcctttatcctcactattttacaacaattctccgcatgtctcgaatccgtcttcaaatctctcaattccggtccacagaagggcgagctcaattcgaagcttgaaggtaagcctatccctaaccctctcctcggtcwcgattctacgcgtaccggtcatcatcaccatcaccat

SEQ ID NO: 61 - protein, 111 aa, Artificial
  amino acid sequence corresponding to canine IL-31 protein with N-terminal truncation (-60N)
MLNSSAILPYFRAIRPLSDKNIIDKIIEQLDKLKFQHEPETEISVPADTFECKSFILTILQQFSACLESVFKSLNSGPQKGELNSKLEGKPIPNPLLGLDSTRTGHHHHHH

SEQ ID NO: 62 - DNA, 333 bp, Artificial
  nucleotide sequence encoding canine IL-31 protein with N-terminal truncation (-60N)
atgcttaactcatcagccattctcccttatttccgtgccattcgccctctttctgataaaaatattattgacaaaattattgaacaactcgacaaattaaaattccaacacgaacccgaaaccgaaatctccgtacctgccgatacctttgaatgcaaatcctttatcctcactattttacaacaattctccgcatgtctcgaatccgtcttcaaatctctcaattccggtccacagaagggcgagctcaattcgaagcttgaaggtaagcctatccctaaccctctcctcggtctcgattctacgcgtaccggtcatcatcaccatcaccat

SEQ ID NO: 63 - protein, 136 aa, Artificial
  amino acid sequence corresponding to canine IL-31 protein with C-terminal truncation at position 20-122
MLELQPLSRGLLEDYQKKETGVPESNRTLLLCLTSDSQPPRLNSSAILPYFRAIRPLSDKNIIDKIIEQLDKLKFQHEPETEISVPADTFECKSFILTILQQFSKGELNSKLEGKPIPNPLLGLDSTRTGHHHHHH

SEQ ID NO: 64 - DNA, 411 bp, Artificial
  nucleotide sequence encoding canine IL-31 protein with C-terminal truncation at position 20-122
atgctcgaattacaacctttatcccgcggtctgctcgaagattaccaaaaaaaagaaacaggcgtcccagaaagcaaccgtacattactcctttgccttacctccgattcccaaccacctcgtcttaactcatcagccattctcccttatttccgtgccattcgccctctttctgataaaaatattattgacaaaattattgaacaactcgacaaattaaaattccaacacgaacccgaaaccgaaatctccgtacctgccgatacctttgaatgcaaatcctttatcctcactattttacaacaattctccaagggcgagctcaattcgaagcttgaaggtaagcctatccctaaccctctcctcggtctcgattctacgcgtaccggtcatcatcaccatcaccattga

SEQ ID NO: 65 - protein, 114 aa, Artificial
  amino acid sequence corresponding to canine IL-31 protein with C-terminal truncation at position 20-100
MLELQPLSRGLLEDYQKKETGVPESNRTLLLCLTSDSQPPRLNSSAILPYFRAIRPLSDKNIIDKIIEQLDKLKFQHEPETEKGELNSKLEGKPIPNPLLGLDSTRTGHHHHHH

SEQ ID NO: 66 - DNA, 345 bp, Artificial
  nucleotide sequence encoding canine IL-31 protein with C-terminal truncation at position 20-100
atgctcgaattacaacctttatcccgcggtctgctcgaagattaccaaaaaaaagaaacaggcgtcccagaaagcaaccgtacattactcctttgccttacctccgattcccaaccacctcgtcttaactcatcagccattctcccttatttccgtgccattcgccctctttctgataaaaatattattgacaaaattattgaacaactcgacaaattaaaattccaacacgaacccgaaaccgaaaagggcgagctcaattcgaagcttgaaggtaagcctatccctaaccctctcctcggtctcgattctacgcgtaccggtcatcatcaccatcaccattga

SEQ ID NO: 67 - protein, 94 aa, Artificial
  amino acid sequence corresponding to canine IL-31 protein with C-terminal truncation at position 20-80
MLELQPLSRGLLEDYQKKETGVPESNRTLLLCLTSDSQPPRLNSSAILPYFRAIRPLSDKNIKGELNSKLEGKPIPNPLLGLDSTRTGHHHHHH

SEQ ID NO: 68 - DNA, 285 bp, Artificial
  nucleotide sequence encoding canine IL-31 protein with C-terminal truncation at position 20-80
atgctcgaattacaacctttatcccgcggtctgctcgaagattaccaaaaaaaagaaacaggcgtcccagaaagcaaccgtacattactcctttgccttacctccgattcccaaccacctcgtcttaactcatcagccattctcccttatttccgtgccattcgccctctttctgataaaaatattaagggcgagctcaattcgaagcttgaaggtaagcctatccctaaccctctcctcggtctcgattctacgcgtaccggtcatcatcaccatcaccattga

SEQ ID NO: 69 - DNA, 444 bp, Felis catus
atgagaggatcccatcaccatcaccaccacggctcatctcatatggcccccgcacatcgcctgcagccgagtgacattcgtaaaattatcttggagctgcgcccgatgtccaagggcttactgcaggattatctgaagaaagagatcgggctgcctgaaagcaaccatagtagcctgccgtgtttatcgtctgatagccagttaccacacatcaatggctctgcgattttgccctactttcgcgccatccgtccgctgtccgataaaaataccatcgacaaaattatcgaacaactggataaattgaagtttcagcgcgagcctgaagcgaaagtttcgatgccagcmgataacttcgaacgcaaaaactttattttagcggtgttgcagcagttttctgcctgtctggaacacgtgctccagtcactcaatagtgggccacaa

SEQ ID NO: 70 - protein, 148 aa, Felis catus
MRGSHHHHHHGSSHMAPAHRLQPSDIRKIILELRPMSKGLLQDYLKKEIGLPESNHSSLPCLSSDSQLPHINGSAILPYFRAIRPLSDKNTIDKIIEQLDKLKFQREPEAKVSMPADNFERKNFILAVLQQFSACLEHVLQSLNSGPQ

SEQ ID NO: 71 - protein, 111 aa, Artificial
  felinized variable light chain mAb sequence, from Mus musculus and Felis catus
EIQMTQSPSSLSASPGDRVTITCKASQSVSFAGTGLMHWYQQKPGKVPKLLIYRASNLEAGVPSRFSGSGSGTDFTLTISSLEPEDAATYYCQQSREYPWTFGQGTKLEIK

SEQ ID NO: 72 - DNA, 333 bp, Artificial
  nucleotide sequence encoding a felinized variable light chain mAb sequence, from Mus musculus and Felis catus
gagattcaaatgacccagagtcctagctcactgagcgcatcacccggggaccgcgtgaccatcacgtgcaaggcatctcagtccgtgtcattcgctggaaccggtctgatgcactggtatcagcaaaaaccagggaaagtccctaaactgctgatctatcgcgcctccaatcttgaggccggggtgccatctcggttctctggtagcggcagcggaactgactttaccctgacaatctcctcactcgagcctgaagacgccgccacctactactgtcaacagtccagagaatacccatggacctttggacagggtaccaagctggagatcaaa

SEQ ID NO: 73 - protein, 118 aa, Artificial
  felinized variable heavy chain mAb sequence, from Mus musculus and Felis catus
DVQLVESGGDLVKPGGSLRLTCVASGFTYSNYGMSWVRQAPGKGLQWVATISYGGSYTYYPDNIKGRFTISRDNAKNTLYLQMNSLKTEDTATYYCVRGYGYDTMDYWGQGTLVTVSS

SEQ ID NO: 74 - DNA, 354 bp, Artificial
  nucleotide sequence encoding a felinized variable heavy chain mAb sequence, from Mus musculus and Felis catus
gacgtgcaactggtcgaaagcggaggcgatcttgtgaagccaggtgggagtctccggctcacatgcgtggcctctggctttacctacagcaactacgggatgagttgggttcgccaggcaccaggaaagggcctgcaatgggtggccactataagctatggtgggtcctatacctactaccctgataatatcaaggggagattcactatttcccgcgacaatgctaagaatactctctacctccagatgaatagcctgaagactgaggataccgctacctactattgcgtgcgcggctacggctacgataccatggactactggggacagggaacccttgtcactgtctcgagc

SEQ ID NO: 75 - protein, 335 aa, Felis catus
ASTTAPSVFPLAPSCGTTSGATVALACLVLGYFPEPVTVSWNSGALTSGVHTFPAVLQASGLYSLSSMVTVPSSRWLSDTFTCNVAHPPSNTKVDKTVRKTDHPPGPKPCDCPKCPPPEMLGGPSIFIFPPKPKDTLSISRTPEVTCLVVDLGPDDSDVQITWFVDNTQVYTAKTSPREEQFNSTYRVVSVLPILHQDWLKGKEFKCKVNSKSLPSPIERTISKAKGQPHEPQVYVLPPAQEELSRNKVSVTCLIKSFHPPDIAVEWEITGQPEPENNYRTTPPQLDSDGTYFVYSKLSVDRSHWQRGNTYTCSVSHEALHSHHTQKSLTQSPGK

SEQ ID NO: 76 - DNA, 1005 bp, Felis catus
gcctccaccacggccccatcggtgttcccactggcccccagctgcgggaccacatctggcgccaccgtggccctggcctgcctggtgttaggctacttccctgagccggtgaccgtgtcctggaactccggcgccctgaccagcggtgtgcacaccttcccggccgtcctgcaggcctcggggctgtactctctcagcagcatggtgacagtgccctccagcaggtggctcagtgacaccttcacctgcaacgtggcccacccgcccagcaacaccaaggtggacaagaccgtgcgcaaaacagaccacccaccgggacccaaaccctgcgactgtcccaaatgcccaccccctgagatgcttggaggaccgtccatcttcatcttccccccaaaacccaaggacaccctctcgatttcccggacgcccgaggtcacatgcttggtggtggacttgggcccagatgactccgatgtccagatcacatggtttgtggataacacccaggtgtacacagccaagacgagtccgcgtgaggagcagttcaacagcacctaccgtgtggtcagtgtcctccccatcctacaccaggactggctcaaggggaaggagttcaagtgcaaggtcaacagcaaatccctcccctcccccatcgagaggaccatctccaaggccaaaggacagccccacgagccccaggtgtacgtcctgcctccagcccaggaggagctcagcaggaacaaagtcagtgtgacctgcctgatcaaatccttccacccgcctgacattgccgtcgagtgggagatcaccggacagccggagccagagaacaactaccggacgaccccgccccagctggacagcgacgggacctacttcgtgtacagcaagctctcggtggacaggtcccactggcagaggggaaacacctacacctgctcggtgtcacacgaagctctgcacagccaccacacacagaaatccctcacccagtctccgggtaaa

SEQ ID NO: 77 - protein, 110 aa, Felis catus
RSDAQPSVFLFQPSLDELHTGSASIVCILNDFYPKEVNVKWKVDGVVQNKGIQESTTEQNSKDSTYSLSSTLTMSSTEYQSHEKFSCEVTHKSLASTLVKSFNRSECQRE

SEQ ID NO: 78 - DNA, 330 bp, Felis catus
cggagtgatgctcagccatctgtctttctcttccaaccatctctggacgagttacatacaggaagtgcctctatcgtgtgcatattgaatgacttctaccccaaagaggtcaatgtcaagtggaaagtggatggcgtagtccaaaacaaaggcatccaggagagcaccacagagcagaacagcaaggacagcacctacagcctcagcagcaccctgacgatgtccagtacggagtaccaaagtcatgaaaagttctcctgcgaggtcactcacaagagcctggcctccaccctcgtcaagagcttcaacaggagcgagtgtcagagagag